European Patent Specification EP 3 971 300 B1, published June 5, 2024. Title: ANALYSIS OF A POLYMER. Applicant: OXFORD NANOPORE TECHNOLOGIES LIMITED. The sequence listing filed with the application follows.

SEQUENCE LISTING (9 sequences)

SEQ ID NO: 1 - DNA, 558 bp, Artificial Sequence
  MS-(B1)8 = MS-(D90N/D91N/D93N/D118R/D134R/E139K)8
atgggtctggataatgaactgagcctggtggacggtcaagatcgtaccctgacggtgcaacaatgggatacctttctgaatggcgtttttccgctggatcgtaatcgcctgacccgtgaatggtttcattccggtcgcgcaaaatatatcgtcgcaggcccgggtgctgacgaattcgaaggcacgctggaactgggttatcagattggctttccgtggtcactgggcgttggtatcaacttctcgtacaccacgccgaatattctgatcaacaatggtaacattaccgcaccgccgtttggcctgaacagcgtgattacgccgaacctgtttccgggtgttagcatctctgcccgtctgggcaatggtccgggcattcaagaagtggcaacctttagtgtgcgcgtttccggcgctaaaggcggtgtcgcggtgtctaacgcccacggtaccgttacgggcgcggccggcggtgtcctgctgcgtccgttcgcgcgcctgattgcctctaccggcgacagcgttacgacctatggcgaaccgtggaatatgaactaa

SEQ ID NO: 2 - protein, 184 aa, Artificial Sequence
  MS-(B1)8 = MS-(D90N/D91N/D93N/D118R/D134R/E139K)8
GLDNELSLVDGQDRTLTVQQWDTFLNGVFPLDRNRLTREWFHSGRAKYIVAGPGADEFEGTLELGYQIGFPWSLGVGINFSYTTPNILINNGNITAPPFGLNSVITPNLFPGVSISARLGNGPGIQEVATFSVRVSGAKGGVAVSNAHGTVTGAAGGVLLRPFARLIASTGDSVTTYGEPWNMN

SEQ ID NO: 3 - DNA, 558 bp, Artificial Sequence
  MS-(B2)8 = MS-(L88N/D90N/D91N/D93N/D118R/D134R/E139K)8
atgggtctggataatgaactgagcctggtggacggtcaagatcgtaccctgacggtgcaacaatgggatacctttctgaatggcgtttttccgctggatcgtaatcgcctgacccgtgaatggtttcattccggtcgcgcaaaatatatcgtcgcaggcccgggtgctgacgaattcgaaggcacgctggaactgggttatcagattggctttccgtggtcactgggcgttggtatcaacttctcgtacaccacgccgaatattaacatcaacaatggtaacattaccgcaccgccgtttggcctgaacagcgtgattacgccgaacctgtttccgggtgttagcatctctgcccgtctgggcaatggtccgggcattcaagaagtggcaacctttagtgtgcgcgtttccggcgctaaaggcggtgtcgcggtgtctaacgcccacggtaccgttacgggcgcggccggcggtgtcctgctgcgtccgttcgcgcgcctgattgcctctaccggcgacagcgttacgacctatggcgaaccgtggaatatgaactaa

SEQ ID NO: 4 - protein, 184 aa, Artificial Sequence
  MS-(B2)8 = MS-(L88N/D90N/D91N/D93N/D118R/D134R/E139K)8
GLDNELSLVDGQDRTLTVQQWDTFLNGVFPLDRNRLTREWFHSGRAKYIVAGPGADEFEGTLELGYQIGFPWSLGVGINFSYTTPNININNGNITAPPFGLNSVITPNLFPGVSISARLGNGPGIQEVATFSVRVSGAKGGVAVSNAHGTVTGAAGGVLLRPFARLIASTGDSVTTYGEPWNMN

SEQ ID NO: 5 - protein, 485 aa, Escherichia coli
MMNDGKQQSTFLFHDYETFGTHPALDRPAQFAAIRTDSEFNVIGEPEVFYCKPADDYLPQPGAVLITGITPQEARAKGENEAAFAARIHSLFTVPKTCILGYNNVRFDDEVTRNIFYRNFYDPYAWSWQHDNSRWDLLDVMRACYALRPEGINWPENDDGLPSFRLEHLTKANGIEHSNAHDAMADVYATIAMAKLVKTRQPRLFDYLFTHRNKHKLMALIDVPQMKPLVHVSGMFGAWRGNTSWVAPLAWHPENRNAVIMVDLAGDISPLLELDSDTLRERLYTAKTDLGDNAAVPVKLVHINKCPVLAQANTLRPEDADRLGINRQHCLDNLKILRENPQVREKVVAIFAEAEPFTPSDNVDAQLYNGFFSDADRAAMKIVLETEPRNLPALDITFVDKRIEKLLFNYRARNFPGTLDYAEQQRWLEHRRQVFTPEFLQGYADELQMLVQQYADDKEKVALLKALWQYAEEIVSGSGHHHHHH

SEQ ID NO: 6 - protein, 268 aa, Escherichia coli
MKFVSFNINGLRARPHQLEAIVEKHQPDVIGLQETKVHDDMFPLEEVAKLGYNVFYHGQKGHYGVALLTKETPIAVRRGFPGDDEEAQRRIIMAEIPSLLGNVTVINGYFPQGESRDHPIKFPAKAQFYQNLQNYLETELKRDNPVLIMGDMNISPTDLDIGIGEENRKRWLRTGKCSFLPEEREWMDRLMSWGLVDTFRHANPQTADRFSWFDYRSKGFDDNRGLRIDLLLASQPLAECCVETGIDYEIRSMEKPSDHAPVWATFRR

SEQ ID NO: 7 - protein, 666 aa, Thermus thermophilus
MRDRVRWRVLSLPPLAQWREVMAALEVGPEAALAYWHRGFRRKEDLDPPLALLPLKGLREAAALLEEALRQGKRIRVHGDYDADGLTGTAILVRGLAALGADVHPFIPHRLEEGYGVLMERVPEHLEASDLFLTVDCGITNHAELRELLENGVEVIVTDHHTPGKTPSPGLVVHPALTPDLKEKPTGAGVVFLLLWALHERLGLPPPLEYADLAAVGTIADVAPLWGWNRALVKEGLARIPASSWVGLRLLAEAVGYTGKAVEVAFRIAPRINAASRLGEAEKALRLLLTDDAAEAQALVGELHRLNARRQTLEEAMLRKLLPQADPEAKAIVLLDPEGHPGVMGIVASRILEATLRPVFLVAQGKGTVRSLAPISAVEALRSAEDLLLRYGGHKEAAGFAMDEALFPAFKARVEAYAARFPDPVREVALLDLLPEPGLLPQVFRELALLEPYGEGNPEPLFLLFGAPEEARRLGEGRHLAFRLKGVRVLAWKQGDLALPPEVEVAGLLSENAWNGHLAYEVQAVDLRKPEALEGGIAPFAYPLPLLEALARARLGEGVYVPEDNPEGLDYARKAGFRLLPPEEAGLWLGLPPRPVLGRRVEVALGREARARLSAPPVLHTPEARLKALVHRRLLFAYERRHPGLFSEALLAYWEVNRVQEPAGSP

SEQ ID NO: 8 - protein, 226 aa, Bacteriophage lambda
MTPDIILQRTGIDVRAVEQGDDAWHKLRLGVITASEVHNVIAKPRSGKKWPDMKMSYFHTLLAEVCTGVAPEVNAKALAWGKQYENDARTLFEFTSGVNVTESPIIYRDESMRTACSPDGLCSDGNGLELKCPFTSRDFMKFRLGGFEAIKSAYMAQVQYSMWVTRKNAWYFANYDPRMKREGLHYVVIERDEKYMASFDEIVPEFIEKMDEALAEIGFVFGEQWR

SEQ ID NO: 9 - protein, 608 aa, Bacteriophage phi-29
MKHMPRKMYSCAFETTTKVEDCRVWAYGYMNIEDHSEYKIGNSLDEFMAWVLKVQADLYFHNLKFDGAFIINWLERNGFKWSADGLPNTYNTIISRMGQWYMIDICLGYKGKRKIHTVIYDSLKKLPFPVKKIAKDFKLTVLKGDIDYHKERPVGYKITPEEYAYIKNDIQIIAEALLIQFKQGLDRMTAGSDSLKGFKDIITTKKFKKVFPTLSLGLDKEVRYAYRGGFTWLNDRFKEKEIGEGMVFDVNSLYPAQMYSRLLPYGEPIVFEGKYVWDEDYPLHIQHIRCEFELKEGYIPTIQIKRSRFYKGNEYLKSSGGEIADLWLSNVDLELMKEHYDLYNVEYISGLKFKATTGLFKDFIDKWTYIKTTSEGAIKQLAKLMLNSLYGKFASNPDVTGKVPYLKENGALGFRLGEEETKDPVYTPMGVFITAWARYTTITAAQACYDRIIYCDTDSIHLTGTEIPDVIKDIVDPKKLGYWAHESTFKRAKYLRQKTYIQDIYMKEVDGKLVEGSPDDYTDIKFSVKCAGMTDKIKKEVTFENFKVGFSRKMKPKPVQVPGGVVLVDDTFTIKSGGSAWSHPQFEKGGGSGGGSGGSAWSHPQFEK